European Patent Application EP 4 209 224 A1, published July 12, 2023. Title: A COMPOSITION FOR IMPROVING INSULIN SENSITIVITY COMPRISING EXTRACT OF GENTIANA TRIFLORA PALLAS. Applicant: MThera Pharma Co., Ltd. apharma. The sequence listing filed with the application follows.

SEQUENCE LISTING (6 sequences)

SEQ ID NO: 1 - RNA, 22 nt, Artificial Sequence
  itih1-qpcr1
tggacacttcagtcaatggtgt

SEQ ID NO: 2 - RNA, 20 nt, Artificial Sequence
  itih1-qpcr2
gatgaaggctgtcttgggga

SEQ ID NO: 3 - RNA, 21 nt, Artificial Sequence
  gapdh-qpcr1
agggctgcttttaactctggt

SEQ ID NO: 4 - RNA, 21 nt, Artificial Sequence
  gapdh-qpcr2
ccccacttgattttggaggga

SEQ ID NO: 5 - RNA, 25 nt, Artificial Sequence
  ogt-qpcr1
ctttagcactctggcaattaaacag

SEQ ID NO: 6 - RNA, 22 nt, Artificial Sequence
  ogt-qpcr2
tcaaataacatgccttggcttc